European Patent Specification EP 3 382 031 B1, published November 29, 2023. Title: Method for producing fibroin-like protein. Applicant: Ajinomoto Co., Inc. SPIBER INC. The sequence listing filed with the application follows.

SEQUENCE LISTING (19 sequences)

SEQ ID NO: 1 - DNA, 3465 bp, Artificial Sequence
  fibroin-like protein gene
  CDS (1)..(3465)
atgcatcaccatcatcatcatcaccaccaccattcctcgggctcatccttggaagtgttatttcaaggaccagcacgagccggttcgggacaacaagggcctggccagcagggcccaggtcaacaagggccaggacagcagggtccttatgggcccggcgcaagcgcagcagctgcggccgctggtggctatggtcctggctccggtcaacagggcccttcgcaacaaggtcccgggcagcaaggtcctggtggccagggtccctacgggccgggggcgagtgcggcagcagccgctgcaggcggttatggtccaggaagcggacagcaaggtccgggaggtcaaggtccgtatggcccaggctctagcgcggctgccgctgccgcgggtggcaacggaccagggagcggacaacagggcgcgggacaacagggtccaggacagcaaggcccaggggcgtcggcggctgcagcggcggccggaggctatggacccggctcaggacaacagggaccgggtcaacaaggacccggtggccaaggcccctatggcccgggcgccagcgcggccgcagccgccgcgggcgggtacggccccggtagcggccagggaccaggtcagcaggggccaggaggtcagggcccatacggtccgggcgcatccgcggcggcggcagcggcaggtggctacggtcccggaagcggccaacaggggccagggcaacaaggaccaggacaacaaggtcctgggggccaaggaccgtatggaccaggagcatcagctgcagccgcggcagctggcggttacggtccaggctacggccagcagggtccgggtcagcagggaccgggaggccaggggccttatggccctggcgcttccgcagccagtgccgcttctggaggatacgggccgggaagcggtcagcaaggccctggccaacaaggacctggaggccaagggccctacggcccaggagcctcggcagccgcagctgccgcaggtgggtatgggccaggtagcgggcaacaagggccgggtcagcaaggaccggggcaacagggacctgggcagcaaggacccgggggtcaaggcccgtacggacctggtgcgtctgcagctgctgctgcggctggtggatatggtccgggatcggggcagcagggtcccggtcagcagggccctggtcagcaagggccaggccaacagggacccggacaacaaggcccgggtcaacagggtcctggacagcaggggccgggccaacaaggccctgggcaacagggtccggggggacagggggcctatgggcctggcgcatctgccgccgctggcgcagccggtgggtacgggcctgggtcaggtcaacaggggcctggtcaacaaggccccgggcaacagggccccggccagcaaggtccagggcagcagggcccgggacagcaagggcctggacaacaggggcccggacagcagggaccttacgggcccggtgcgagcgcagcggccgccgccgcagggggatatggccccggatcgggccagcagggaccaggccagcaaggacctggccaacagggcccggggggtcaggggccgtatggtcccggcgctgcaagtgctgcagtgtccgtttctagagcacgagccggttcgggacaacaagggcctggccagcagggcccaggtcaacaagggccaggacagcagggtccttatgggcccggcgcaagcgcagcagctgcggccgctggtggctatggtcctggctccggtcaacagggcccttcgcaacaaggtcccgggcagcaaggtcctggtggccagggtccctacgggccgggggcgagtgcggcagcagccgctgcaggcggttatggtccaggaagcggacagcaaggtccgggaggtcaaggtccgtatggcccaggctctagcgcggctgccgctgccgcgggtggcaacggaccagggagcggacaacagggcgcgggacaacagggtccaggacagcaaggcccaggggcgtcggcggctgcagcggcggccggaggctatggacccggctcaggacaacagggaccgggtcaacaaggacccggtggccaaggcccctatggcccgggcgccagcgcggccgcagccgccgcgggcgggtacggccccggtagcggccagggaccaggtcagcaggggccaggaggtcagggcccatacggtccgggcgcatccgcggcggcggcagcggcaggtggctacggtcccggaagcggccaacaggggccagggcaacaaggaccaggacaacaaggtcctgggggccaaggaccgtatggaccaggagcatcagctgcagccgcggcagctggcggttacggtccaggctacggccagcagggtccgggtcagcagggaccgggaggccaggggccttatggccctggcgcttccgcagccagtgccgcttctggaggatacgggccgggaagcggtcagcaaggccctggccaacaaggacctggaggccaagggccctacggcccaggagcctcggcagccgcagctgccgcaggtgggtatgggccaggtagcgggcaacaagggccgggtcagcaaggaccggggcaacagggacctgggcagcaaggacccgggggtcaaggcccgtacggacctggtgcgtctgcagctgctgctgcggctggtggatatggtccgggatcggggcagcagggtcccggtcagcagggccctggtcagcaagggccaggccaacagggacccggacaacaaggcccgggtcaacagggtcctggacagcaggggccgggccaacaaggccctgggcaacagggtccggggggacagggggcctatgggcctggcgcatctgccgccgctggcgcagccggtgggtacgggcctgggtcaggtcaacaggggcctggtcaacaaggccccgggcaacagggccccggccagcaaggtccagggcagcagggcccgggacagcaagggcctggacaacaggggcccggacagcagggaccttacgggcccggtgcgagcgcagcggccgccgccgcagggggatatggccccggatcgggccagcagggaccaggccagcaaggacctggccaacagggcccggggggtcaggggccgtatggtcccggcgctgcaagtgctgcagtgtccgttggaggttacggccctcagtcttcgtctgttccggtggcgtccgcagttgcgagtagactgtcttcacctgctgcttcatcgcgagtatcgagcgctgtttcgtctcttgtctcgtcgggtcccacgaaacatgccgccctttcaaatacgatttcatctgtagtgtcccaagttagtgcaagtaacccggggttatccggatgcgacgttctcgttcaggcactcctagaagtagtatccgcgttggtgagcatcttataa

SEQ ID NO: 2 - protein, 1154 aa, Artificial Sequence
  Synthetic Construct
MHHHHHHHHHHSSGSSLEVLFQGPARAGSGQQGPGQQGPGQQGPGQQGPYGPGASAAAAAAGGYGPGSGQQGPSQQGPGQQGPGGQGPYGPGASAAAAAAGGYGPGSGQQGPGGQGPYGPGSSAAAAAAGGNGPGSGQQGAGQQGPGQQGPGASAAAAAAGGYGPGSGQQGPGQQGPGGQGPYGPGASAAAAAAGGYGPGSGQGPGQQGPGGQGPYGPGASAAAAAAGGYGPGSGQQGPGQQGPGQQGPGGQGPYGPGASAAAAAAGGYGPGYGQQGPGQQGPGGQGPYGPGASAASAASGGYGPGSGQQGPGQQGPGGQGPYGPGASAAAAAAGGYGPGSGQQGPGQQGPGQQGPGQQGPGGQGPYGPGASAAAAAAGGYGPGSGQQGPGQQGPGQQGPGQQGPGQQGPGQQGPGQQGPGQQGPGQQGPGGQGAYGPGASAAAGAAGGYGPGSGQQGPGQQGPGQQGPGQQGPGQQGPGQQGPGQQGPGQQGPYGPGASAAAAAAGGYGPGSGQQGPGQQGPGQQGPGGQGPYGPGAASAAVSVSRARAGSGQQGPGQQGPGQQGPGQQGPYGPGASAAAAAAGGYGPGSGQQGPSQQGPGQQGPGGQGPYGPGASAAAAAAGGYGPGSGQQGPGGQGPYGPGSSAAAAAAGGNGPGSGQQGAGQQGPGQQGPGASAAAAAAGGYGPGSGQQGPGQQGPGGQGPYGPGASAAAAAAGGYGPGSGQGPGQQGPGGQGPYGPGASAAAAAAGGYGPGSGQQGPGQQGPGQQGPGGQGPYGPGASAAAAAAGGYGPGYGQQGPGQQGPGGQGPYGPGASAASAASGGYGPGSGQQGPGQQGPGGQGPYGPGASAAAAAAGGYGPGSGQQGPGQQGPGQQGPGQQGPGGQGPYGPGASAAAAAAGGYGPGSGQQGPGQQGPGQQGPGQQGPGQQGPGQQGPGQQGPGQQGPGQQGPGGQGAYGPGASAAAGAAGGYGPGSGQQGPGQQGPGQQGPGQQGPGQQGPGQQGPGQQGPGQQGPYGPGASAAAAAAGGYGPGSGQQGPGQQGPGQQGPGGQGPYGPGAASAAVSVGGYGPQSSSVPVASAVASRLSSPAASSRVSSAVSSLVSSGPTKHAALSNTISSVVSQVSASNPGLSGCDVLVQALLEVVSALVSIL

SEQ ID NO: 3 - protein, 636 aa, Araneus diadematus
ARAGSGQQGPGQQGPGQQGPGQQGPYGPGASAAAAAAGGYGPGSGQQGPSQQGPGQQGPGGQGPYGPGASAAAAAAGGYGPGSGQQGPGGQGPYGPGSSAAAAAAGGNGPGSGQQGAGQQGPGQQGPGASAAAAAAGGYGPGSGQQGPGQQGPGGQGPYGPGASAAAAAAGGYGPGSGQGPGQQGPGGQGPYGPGASAAAAAAGGYGPGSGQQGPGQQGPGQQGPGGQGPYGPGASAAAAAAGGYGPGYGQQGPGQQGPGGQGPYGPGASAASAASGGYGPGSGQQGPGQQGPGGQGPYGPGASAAAAAAGGYGPGSGQQGPGQQGPGQQGPGQQGPGGQGPYGPGASAAAAAAGGYGPGSGQQGPGQQGPGQQGPGQQGPGQQGPGQQGPGQQGPGQQGPGQQGPGGQGAYGPGASAAAGAAGGYGPGSGQQGPGQQGPGQQGPGQQGPGQQGPGQQGPGQQGPGQQGPYGPGASAAAAAAGGYGPGSGQQGPGQQGPGQQGPGGQGPYGPGAASAAVSVGGYGPQSSSVPVASAVASRLSSPAASSRVSSAVSSLVSSGPTKHAALSNTISSVVSQVSASNPGLSGCDVLVQALLEVVSALVSILGSSSIGQINYGASAQYTQMVGQSVAQALA

SEQ ID NO: 4 - DNA, 2190 bp, Araneus diadematus
agatatacataatgcaccaccatcaccaccatcatcaccatcatagcagcggcagcagcctggaagttctgtttcagggtccggcgcgtgcgggtagcggccagcagggcccgggtcagcagggtccgggccaacaaggtccgggccagcagggcccgtatggtccgggtgcaagcgcagcagcagcggccgcaggcggttacggcccgggtagcggccagcagggcccgagccagcagggcccgggccagcagggtccgggcggtcagggtccgtacggtccgggcgcgagcgcggccgccgcggccgcaggcggttacgggccgggcagcggtcagcagggcccgggcggtcagggcccgtatggcccgggtagcagcgcggccgcggcggccgcaggcggtaatggtccgggcagcggccagcagggtgcgggccaacaaggcccgggtcagcagggcccgggtgccagcgccgccgcagcggccgcaggcggttacggtccgggtagcggtcagcagggtcctggccaacaaggcccgggcggtcaaggtccttacggcccgggcgccagcgccgcggctgcggccgcaggcggttacggaccgggtagcggccagggtcctggtcaacaaggtccgggcggtcaaggcccgtatggtccgggcgccagcgcggcggccgcggccgcaggcggttacgggccaggtagcggccagcagggtcctggccagcagggtcctggacaacaaggaccgggcggtcaaggaccgtacggcccgggcgcgagcgccgcggcagcggccgcaggcggttatggtccgggttacggtcagcagggtcccggtcaacagggaccgggcggtcaaggtccgtatggcccgggtgcgagcgcggccagcgcagcgagcggcggttacggtcctggttctggtcagcagggtcctggacagcaaggtccgggcggtcagggaccttacggtccgggtgcgagcgccgcagcggccgcagcgggcggttacggccctggctctggtcagcagggtccaggtcaacagggtcctggtcaacagggtcccggtcagcaaggcccgggcggtcagggtccttatggtccgggcgcaagcgcggccgccgccgcagcgggcggttacggtcctggcagtggtcagcagggtccgggacaacagggtcctggacagcagggtcctgggcagcagggtcctggtcagcaaggtcctggtcagcagggccctggccagcagggtcccggtcagcagggccctggtcaacaaggaccgggcggtcagggcgcgtatggtccgggtgccagcgccgcagcgggcgccgcaggcggttacgggcctggtagtggtcaacaggggcctggccaacagggccctggtcagcaaggccctggtcaacagggccctggtcagcagggccccggtcaacagggccccggtcaacagggtccaggtcagcaaggtccgtacggcccgggcgcaagcgccgcggcagcggccgcaggcggttacgggcccggctctggtcaacaggggcccggtcaacagggcccaggtcaacaggggccgggcggtcaagggccttatggcccgggcgccgcgagcgccgccgtgagcgttggcggttacggtccgcagagcagcagcgtgccggttgccagcgcagtggccagccgcctgagcagcccggccgcgagcagccgtgtgagcagcgcagttagcagcttagtgagcagcggtccgaccaaacatgccgcgctgagcaacacgattagcagcgtggttagccaggtttctgcaagcaatccgggtctgagcggttgcgatgtgctggttcaggcgctgctggaagtggttagcgccttagtgagcatcctgggcagcagcagcattggccagatcaattatggcgcgagcgcccagtacacccagatggttggtcagagcgtggcacaggccctggcgtgaaattcgagctccgtcgacaagcttgcggccgcactcgagcaccaccaccaccaccactgagatccggctgctaacaaagcccgaaaggaagctgagttggctgctgccaccgctgagcaataactagcataaccccttggggcctctaaacgggtcttgaggggttttttgctgaaaggaggaactatatccggat

SEQ ID NO: 5 - protein, 660 aa, Araneus diadematus
MHHHHHHHHHHSSGSSLEVLFQGPARAGSGQQGPGQQGPGQQGPGQQGPYGPGASAAAAAAGGYGPGSGQQGPSQQGPGQQGPGGQGPYGPGASAAAAAAGGYGPGSGQQGPGGQGPYGPGSSAAAAAAGGNGPGSGQQGAGQQGPGQQGPGASAAAAAAGGYGPGSGQQGPGQQGPGGQGPYGPGASAAAAAAGGYGPGSGQGPGQQGPGGQGPYGPGASAAAAAAGGYGPGSGQQGPGQQGPGQQGPGGQGPYGPGASAAAAAAGGYGPGYGQQGPGQQGPGGQGPYGPGASAASAASGGYGPGSGQQGPGQQGPGGQGPYGPGASAAAAAAGGYGPGSGQQGPGQQGPGQQGPGQQGPGGQGPYGPGASAAAAAAGGYGPGSGQQGPGQQGPGQQGPGQQGPGQQGPGQQGPGQQGPGQQGPGQQGPGGQGAYGPGASAAAGAAGGYGPGSGQQGPGQQGPGQQGPGQQGPGQQGPGQQGPGQQGPGQQGPYGPGASAAAAAAGGYGPGSGQQGPGQQGPGQQGPGGQGPYGPGAASAAVSVGGYGPQSSSVPVASAVASRLSSPAASSRVSSAVSSLVSSGPTKHAALSNTISSVVSQVSASNPGLSGCDVLVQALLEVVSALVSILGSSSIGQINYGASAQYTQMVGQSVAQALA

SEQ ID NO: 6 - DNA, 65 bp, Escherichia coli
ctgttgacaattaatcatcgaactagttaactagtacgcaagttcacgtaaaaagggtatcgaca

SEQ ID NO: 7 - DNA, 132 bp, Escherichia coli
tcaggtggcacttttcggggaaatgtgcgcggaacccctatttgtttatttttctaaatacattcaaatatgtatccgctcatgagacaataaccctgataaatgcttcaataatattgaaaaaggaagagt

SEQ ID NO: 8 - DNA, 327 bp, Escherichia coli
atggcccaacaatcaccctattcagcagcgatggcagaacagcgtcaccaggagtggttacgttttgtcgacctgcttaagaatgcctaccaaaacgatctccatttaccgttgttaaacctgatgctgacgccagatgagcgcgaagcgttggggactcgcgtgcgtattgtcgaagagctgttgcgcggcgaaatgagccagcgtgagttaaaaaatgaactcggcgcaggcatcgcgacgattacgcgtggatctaacagcctgaaagccgcgcccgtcgagctgcgccagtggctggaagaggtgttgctgaaaagcgattga

SEQ ID NO: 9 - protein, 108 aa, Escherichia coli
MAQQSPYSAAMAEQRHQEWLRFVDLLKNAYQNDLHLPLLNLMLTPDEREALGTRVRIVEELLRGEMSQRELKNELGAGIATITRGSNSLKAAPVELRQWLEEVLLKSD

SEQ ID NO: 10 - DNA, 58 bp, Artificial Sequence
  primer
aatgagcgggcttttttttgaacaaaattagagaataacatgaagcctgcttttttat

SEQ ID NO: 11 - DNA, 58 bp, Artificial Sequence
  primer
gaaagttaaaatgccgccagcggaactggcggctgtgggacgctcaagttagtataaa

SEQ ID NO: 12 - DNA, 1551 bp, Artificial Sequence
  attL-Kmr-attL sequence
ctagacgctcaagttagtataaaaaagctgaacgagaaacgtaaaatgatataaatatcaatatattaaattagattttgcataaaaaacagactacataatactgtaaaacacaacatatgcagtcactatgaatcaactacttagatggtattagtgacctgtaacagactgcaggggggggggggaaagccacgttgtgtctcaaaatctctgatgttacattgcacaagataaaaatatatcatcatgaacaataaaactgtctgcttacataaacagtaatacaaggggtgttatgagccatattcaacgggaaacgtcttgctcgaggccgcgattaaattccaacatggatgctgatttatatgggtataaatgggctcgcgataatgtcgggcaatcaggtgcgacaatctatcgattgtatgggaagcccgatgcgccagagttgtttctgaaacatggcaaaggtagcgttgccaatgatgttacagatgagatggtcagactaaactggctgacggaatttatgcctcttccgaccatcaagcattttatccgtactcctgatgatgcatggttactcaccactgcgatccccgggaaaacagcattccaggtattagaagaatatcctgattcaggtgaaaatattgttgatgcgctggcagtgttcctgcgccggttgcattcgattcctgtttgtaattgtccttttaacagcgatcgcgtatttcgtctcgctcaggcgcaatcacgaatgaataacggtttggttgatgcgagtgattttgatgacgagcgtaatggctggcctgttgaacaagtctggaaagaaatgcataagcttttgccattctcaccggattcagtcgtcactcatggtgatttctcacttgataaccttatttttgacgaggggaaattaataggttgtattgatgttggacgagtcggaatcgcagaccgataccaggatcttgccatcctatggaactgcctcggtgagttttctccttcattacagaaacggctttttcaaaaatatggtattgataatcctgatatgaataaattgcagtttcatttgatgctcgatgagtttttctaatcagaattggttaattggttgtaacactggcagagcattacgctgacttgacgggacggcggctttgttgaataaatcgaacttttgctgagttgaaggatcagatcacgcatcttcccgacaacgcagaccgttccgtggcaaagcaaaagttcaaaatcaccaactggtccacctacaacaaagctctcatcaaccgtggctccctcactttctggctggatgatggggcgattcaggcctggtatgagtcagcaacaccttcttcacgaggcagacctcagcgccccccccccctgcaggtcgacggatccggggaattcgaaatcaaataatgattttattttgactgatagtgacctgttcgttgcaacaaattgataagcaatgcttttttataatgccaacttagtataaaaaagcaggcttcaagatct

SEQ ID NO: 13 - DNA, 54 bp, Artificial Sequence
  primer
tagaggatcgagatcctgttgacaattaatcatcgaactagttaactagtacgc

SEQ ID NO: 14 - DNA, 62 bp, Artificial Sequence
  primer
tgatggtgatgcatatgtcgataccctttttacgtgaacttgcgtactagttaactagttcg

SEQ ID NO: 15 - DNA, 50 bp, Artificial Sequence
  primer
aatattgaaaaaggaagagtatggcccaacaatcaccctattcagcagcg

SEQ ID NO: 16 - DNA, 45 bp, Artificial Sequence
  primer
taagtgcggcgacgaatcatgcctaccaaacatattgaaattacg

SEQ ID NO: 17 - DNA, 80 bp, Artificial Sequence
  primer
aatacattcaaatatgtatccgctcatgagacaataaccctgataaatgcttcaataatattgaaaaaggaagagtatgg

SEQ ID NO: 18 - DNA, 80 bp, Artificial Sequence
  primer
gtcaggtggcacttttcggggaaatgtgcgcggaacccctatttgtttatttttctaaatacattcaaatatgtatccgc

SEQ ID NO: 19 - DNA, 43 bp, Artificial Sequence
  primer
ggcgccatctccttgtcaggtggcacttttcggggaaatgtgc